European Patent Application EP 4 682 142 A1, published January 21, 2026. Title: 1H-PYRROLE-2-AMIDE DERIVATIVE AND USE THEREOF. Applicant: CHONGQING PHARSCIN INNOBIO CO., LTD. Application EP. The sequence listing filed with the application follows.

SEQUENCE LISTING (1 sequence)

SEQ ID NO: 1 - RNA, 17 nt, synthetic construct
  source 1..17: mol_type = other RNA
aagaaccggactaagct